European Patent Specification EP 3 640 258 B1, published May 27, 2026. Title: Novel polypeptide and a method for producing putrescine using the same. Applicant: CJ CheilJedang Corporation. The sequence listing filed with the application follows.

SEQUENCE LISTING (22 sequences)

SEQ ID NO: 1 - protein, 494 aa, Artificial Sequence
  ATCC13032 NCgl2522
MTSETLQAQAPTKTQRWAFLAVISGGLFLIGVDNSILYTALPLLREQLAATETQALWIINAYPLLMAGLLLGTGTLGDKIGHRRMFLMGLSIFGIASLGAAFAPTAWALVAARAFLGIGAATMMPATLALIRITFEDERERNTAIGIWGSVAILGAAAGPIIGGALLEFFWWGSVFLINVPVAVIALIATLFVAPANIANPSKHWDFLSSFYALLTLAGLIITIKESVNTARHMPLLLGAVIMLIIGAVLFSSRQKKIEEPLLDLSLFRNRLFLGGVVAAGMAMFTVSGLEMTTSQRFQLSVGFTPLEAGLLMIPAALGSFPMSIIGGANLHRWGFKPLISGGFAATAVGIALCIWGATHTDGLPFFIAGLFFMGAGAGSVMSVSSTAIIGSAPVRKAGMASSIEEVSYEFGTLLSVAILGSLFPFFYSLHAPAEVADNFSAGVHHAIDGDAARASLDTAYINVLIIALVCAVAAALISSYLFRGNPKGANNAH

SEQ ID NO: 2 - protein, 494 aa, Artificial Sequence
  ATCC13869 NCgl2522
MISETLQAQAPTKTQRWAFLAVISGGLFLIGVDNSILYTALPLLREQLAATETQALWIINAYPLLMAGLLLGTGTLGDKIGHRRMFLMGLSIFGIASLGAAFAPTAWALVAARAFLGIGAATMMPATLALIRITFEDERERNTAIGIWGSVAILGAAAGPIIGGALLEFFWWGSVFLINVPVAVIALIATLFVAPANIANPSKHWDFLSSFYALLTLAGLIVTIKESVNTARHLPLLVGAIILLIIGAVLFSSRQKKIEEPLLDLSLFRNRLFLGGVVAAGMAMFTVSGLEMTTSQRFQLSVGFTPLEAGLLMIPAALGSFPMSIIGGANLHRWGFKPLISGGFLATAVGIALCIWGATHTDGLPFFIAGLFFMGAGAGSVMSVSSTAIIGSAPVRKAGMASSIEEVSYEFGTLLSVAILGSLFPFFYSLHAPAEVADNFSAGVHHAIYGDAARASLDTAYINVLIIALVCAVAAALISSYLFRGNPKGANNAH

SEQ ID NO: 3 - protein, 494 aa, Artificial Sequence
  NCgl2522_G77A (ATCC13032)
MTSETLQAQAPTKTQRWAFLAVISGGLFLIGVDNSILYTALPLLREQLAATETQALWIINAYPLLMAGLLLGTGTLADKIGHRRMFLMGLSIFGIASLGAAFAPTAWALVAARAFLGIGAATMMPATLALIRITFEDERERNTAIGIWGSVAILGAAAGPIIGGALLEFFWWGSVFLINVPVAVIALIATLFVAPANIANPSKHWDFLSSFYALLTLAGLIITIKESVNTARHMPLLLGAVIMLIIGAVLFSSRQKKIEEPLLDLSLFRNRLFLGGVVAAGMAMFTVSGLEMTTSQRFQLSVGFTPLEAGLLMIPAALGSFPMSIIGGANLHRWGFKPLISGGFAATAVGIALCIWGATHTDGLPFFIAGLFFMGAGAGSVMSVSSTAIIGSAPVRKAGMASSIEEVSYEFGTLLSVAILGSLFPFFYSLHAPAEVADNFSAGVHHAIDGDAARASLDTAYINVLIIALVCAVAAALISSYLFRGNPKGANNAH

SEQ ID NO: 4 - protein, 494 aa, Artificial Sequence
  NCgl2522_G77R (ATCC13032)
MTSETLQAQAPTKTQRWAFLAVISGGLFLIGVDNSILYTALPLLREQLAATETQALWIINAYPLLMAGLLLGTGTLRDKIGHRRMFLMGLSIFGIASLGAAFAPTAWALVAARAFLGIGAATMMPATLALIRITFEDERERNTAIGIWGSVAILGAAAGPIIGGALLEFFWWGSVFLINVPVAVIALIATLFVAPANIANPSKHWDFLSSFYALLTLAGLIITIKESVNTARHMPLLLGAVIMLIIGAVLFSSRQKKIEEPLLDLSLFRNRLFLGGVVAAGMAMFTVSGLEMTTSQRFQLSVGFTPLEAGLLMIPAALGSFPMSIIGGANLHRWGFKPLISGGFAATAVGIALCIWGATHTDGLPFFIAGLFFMGAGAGSVMSVSSTAIIGSAPVRKAGMASSIEEVSYEFGTLLSVAILGSLFPFFYSLHAPAEVADNFSAGVHHAIDGDAARASLDTAYINVLIIALVCAVAAALISSYLFRGNPKGANNAH

SEQ ID NO: 5 - protein, 494 aa, Artificial Sequence
  NCgl2522_G77A (ATCC13869)
MISETLQAQAPTKTQRWAFLAVISGGLFLIGVDNSILYTALPLLREQLAATETQALWIINAYPLLMAGLLLGTGTLADKIGHRRMFLMGLSIFGIASLGAAFAPTAWALVAARAFLGIGAATMMPATLALIRITFEDERERNTAIGIWGSVAILGAAAGPIIGGALLEFFWWGSVFLINVPVAVIALIATLFVAPANIANPSKHWDFLSSFYALLTLAGLIVTIKESVNTARHLPLLVGAIILLIIGAVLFSSRQKKIEEPLLDLSLFRNRLFLGGVVAAGMAMFTVSGLEMTTSQRFQLSVGFTPLEAGLLMIPAALGSFPMSIIGGANLHRWGFKPLISGGFLATAVGIALCIWGATHTDGLPFFIAGLFFMGAGAGSVMSVSSTAIIGSAPVRKAGMASSIEEVSYEFGTLLSVAILGSLFPFFYSLHAPAEVADNFSAGVHHAIYGDAARASLDTAYINVLIIALVCAVAAALISSYLFRGNPKGANNAH

SEQ ID NO: 6 - protein, 494 aa, Artificial Sequence
  NCgl2522_G77R (ATCC13869)
MISETLQAQAPTKTQRWAFLAVISGGLFLIGVDNSILYTALPLLREQLAATETQALWIINAYPLLMAGLLLGTGTLRDKIGHRRMFLMGLSIFGIASLGAAFAPTAWALVAARAFLGIGAATMMPATLALIRITFEDERERNTAIGIWGSVAILGAAAGPIIGGALLEFFWWGSVFLINVPVAVIALIATLFVAPANIANPSKHWDFLSSFYALLTLAGLIVTIKESVNTARHLPLLVGAIILLIIGAVLFSSRQKKIEEPLLDLSLFRNRLFLGGVVAAGMAMFTVSGLEMTTSQRFQLSVGFTPLEAGLLMIPAALGSFPMSIIGGANLHRWGFKPLISGGFLATAVGIALCIWGATHTDGLPFFIAGLFFMGAGAGSVMSVSSTAIIGSAPVRKAGMASSIEEVSYEFGTLLSVAILGSLFPFFYSLHAPAEVADNFSAGVHHAIYGDAARASLDTAYINVLIIALVCAVAAALISSYLFRGNPKGANNAH

SEQ ID NO: 7 - DNA, 36 bp, Artificial Sequence
  13032-putE-EF-FX
ccggggatcctctagaacttcagaaaccttacaggc

SEQ ID NO: 8 - DNA, 36 bp, Artificial Sequence
  13032-putE-EF-RX
gcaggtcgactctagactagtgcgcattattggctc

SEQ ID NO: 9 - DNA, 24 bp, Artificial Sequence
  SM_putE_G77-F
ccggcactttgnnkgacaaaatcg

SEQ ID NO: 10 - DNA, 24 bp, Artificial Sequence
  SM_putE_G77-R
cgattttgtcmnncaaagtgccgg

SEQ ID NO: 11 - DNA, 34 bp, Artificial Sequence
  pDC-Pself-putE-up-FX
ccggggatcctctagacctctaagcgcctcaaag

SEQ ID NO: 12 - DNA, 34 bp, Artificial Sequence
  pDC-putE-up-RX
gcaggtcgactctagagattcgcgatattggccg

SEQ ID NO: 13 - DNA, 24 bp, Artificial Sequence
  putE-G77A-F
ccggcactttggctgacaaaatcg

SEQ ID NO: 14 - DNA, 24 bp, Artificial Sequence
  putE-G77A-R
cgattttgtcagccaaagtgccgg

SEQ ID NO: 15 - DNA, 24 bp, Artificial Sequence
  putE-G77R-F
ccggcactttgcgtgacaaaatcg

SEQ ID NO: 16 - DNA, 24 bp, Artificial Sequence
  putE-G77R-R
cgattttgtcacgcaaagtgccgg

SEQ ID NO: 17 - DNA, 37 bp, Artificial Sequence
  NCgl2522-L5
tgcaggtcgactctagagttctgcgtagctgtgtgcc

SEQ ID NO: 18 - DNA, 31 bp, Artificial Sequence
  NCgl2522-L3
gatgtttctggatcgtaactgtaacgaatgg

SEQ ID NO: 19 - DNA, 24 bp, Artificial Sequence
  CJ7-F
agaaacatcccagcgctactaata

SEQ ID NO: 20 - DNA, 23 bp, Artificial Sequence
  CJ7-R
agtgtttcctttcgttgggtacg

SEQ ID NO: 21 - DNA, 41 bp, Artificial Sequence
  NCgl2522-R5
caacgaaaggaaacactatgatttcagaaactttgcaggcg

SEQ ID NO: 22 - DNA, 40 bp, Artificial Sequence
  NCgl2522-R3
tcggtacccggggatcccacaaaaagcgtagcgatcaacg